European Patent Application EP 4 265 634 A2, published October 25, 2023. Title: Enhancer of T cells or B cells with memory function, inhibitor of malignant tumor recurrence, and inducerr of T cells or B cells with memory function. Applicant: YAMAGUCHI UNIVERSITY. Application EP. The sequence listing filed with the application follows.

SEQUENCE LISTING (15 sequences)

SEQ ID NO: 1 - protein, 177 aa, synthetic construct
  REGION 1..177: note = human IL-7 AA
MFHVSFRYIFGLPPLILVLLPVASSDCDIEGKDGKQYESVLMVSIDQLLDSMKEIGSNCLNNEFNFFKRHICDANKEGMFLFRAARKLRQFLKMNSTGDFDLHLLKVSEGTTILLNCTGQVKGRKPAALGEAQPTKSLEENKSLKEQKKLNDLCFLKRLLQEIKTCWNKILMGTKEH

SEQ ID NO: 2 - protein, 98 aa, synthetic construct
  REGION 1..98: note = human CCL19 AA
MALLLALSLLVLWTSPAPTLSGTNDAEDCCLSVTQKPIPGYIVRNFHYLLIKDGCRVPAVVFTTLRGRQLCAPPDQPWVERIIQRLQRTSAKMKRRSS

SEQ ID NO: 3 - protein, 128 aa, synthetic construct
  REGION 1..128: note = VH07_aa
QVQLQQSGPGLVTPSQTLSLTCAISGDSVSSNSATWNWIRQSPSRGLEWLGRTYYRSKWYNDYAVSVKSRMSINPDTSKNQFSLQLNSVTPEDTAVYYCARGMMTYYYGMDVWGQGTTVTVSSGILGS

SEQ ID NO: 4 - protein, 15 aa, synthetic construct
  REGION 1..15: note = linker 15_aa
GGGGSGGGGSGGGGS

SEQ ID NO: 5 - protein, 116 aa, synthetic construct
  REGION 1..116: note = VL07_aa
QPVLTQSSSLSASPGASASLTCTLRSGINVGPYRIYWYQQKPGSPPQYLLNYKSDSDKQQGSGVPSRFSGSKDASANAGVLLISGLRSEDEADYYCMIWHSSAAVFGGGTQLTVLS

SEQ ID NO: 6 - protein, 283 aa, synthetic construct
  REGION 1..283: note = hCD8-hCD28-h4-1BB-hCD3
FVPVFLPAKPTTTPAPRPPTPAPTIASQPLSLRPEACRPAAGGAVHTRGLDFACDIYIWAPLAGTCGVLLLSLVITLYCNHRNRSKRSRLLHSDYMNMTPRRPGPTRKHYQPYAPPRDFAAYRSRFSVVKRGRKKLLYIFKQPFMRPVQTTQEEDGCSCRFPEEEEGGCELRVKFSRSADAPAYQQGQNQLYNELNLGRREEYDVLDKRRGRDPEMGGKPRRKNPQEGLYNELQKDKMAEAYSEIGMKGERRRGKGHDGLYQGLSTATKDTYDALHMQALPPR

SEQ ID NO: 7 - protein, 25 aa, synthetic construct
  REGION 1..25: note = F2A_aa
GSGVKQTLNFDLLKLAGDVESNPGP

SEQ ID NO: 8 - protein, 19 aa, synthetic construct
  REGION 1..19: note = signal peptide_aa
MDWTWRILFLVAAATGAHS

SEQ ID NO: 9 - DNA, 1665 bp, synthetic construct
  misc_feature 1..1665: note = Mouse Il-7-F2A-mouseCCL19-F2A-eGFP
  source 1..1665: mol_type = other DNA
atggtccacgtctccttcagatacatcttcggcatcccccccctgatcctggtcctcctgcctgtcacctccagcgaatgtcatatcaaggacaaagagggcaaggcttatgagagcgtcctgatgatctccattgatgagctggataagatgaccggcaccgacagcaactgtcccaacaatgagcccaacttctttagaaagcacgtgtgtgacgataccaaggaggctgccttcctgaacagggccgccagaaagctgaagcagttcctgaagatgaacatttccgaggagttcaacgtgcacctcctcaccgtgagccagggcacccagacactggtcaattgcacctccaaggaggagaagaacgtgaaagagcagaaaaagaatgatgcttgtttcctcaagaggctgctgagggagatcaagacctgttggaataagatcctgaaaggcagcatcggcagcggagtcaagcaaaccctgaacttcgacctgctgaaactggccggagatgtggagagcaatcccggccctatggcccccagagtcacccctctgctggccttcagcctgctcgtgctgtggaccttccccgctcccaccctgggcggcgccaatgatgctgaggactgttgcctctccgtgacccagaggcccatccctggaaacatcgtcaaagccttcaggtacctgctcaacgaagacggatgtagggtgcctgccgtggtgttcacaacactgagaggctaccagctctgcgcccctcctgatcagccctgggtcgacagaatcatcagaaggctgaagaagtccagcgccaagaacaaaggcaatagcacaaggagaagccctgtgagcgaattcggaagcggagtgaaacagactttgaattttgaccttctcaagttggcgggagacgtggagtccaaccctggaccatgcatggtgagcaagggcgaggagctgttcaccggggtggtgcccatcctggtcgagctggacggcgacgtaaacggccacaagttcagcgtgtccggcgagggcgagggcgatgccacctacggcaagctgaccctgaagttcatctgcaccaccggcaagctgcccgtgccctggcccaccctcgtgaccaccctgacctacggcgtgcagtgcttcagccgctaccccgaccacatgaagcagcacgacttcttcaagtccgccatgcccgaaggctacgtccaggagcgcaccatcttcttcaaggacgacggcaactacaagacccgcgccgaggtgaagttcgagggcgacaccctggtgaaccgcatcgagctgaagggcatcgacttcaaggaggacggcaacatcctggggcacaagctggagtacaactacaacagccacaacgtctatatcatggccgacaagcagaagaacggcatcaaggtgaacttcaagatccgccacaacatcgaggacggcagcgtgcagctcgccgaccactaccagcagaacacccccatcggcgacggccccgtgctgctgcccgacaaccactacctgagcacccagtccgccctgagcaaagaccccaacgagaagcgcgatcacatggtcctgctggagttcgtgaccgccgccgggatcactctcggcatggacgagctgtacaagtaa

SEQ ID NO: 10 - DNA, 37 bp, synthetic construct
  misc_feature 1..37: note = primer
  source 1..37: mol_type = other DNA
atggccggaccggccaccggtcgccaccatgagcgag

SEQ ID NO: 11 - DNA, 41 bp, synthetic construct
  misc_feature 1..41: note = primer
  source 1..41: mol_type = other DNA
tcgaattcgctagcggccgcttaattaagcttgtgccccag

SEQ ID NO: 12 - DNA, 33 bp, synthetic construct
  misc_feature 1..33: note = primer
  source 1..33: mol_type = other DNA
gctccggacgccaccatggaagatgccaaaaac

SEQ ID NO: 13 - DNA, 31 bp, synthetic construct
  misc_feature 1..31: note = primer
  source 1..31: mol_type = other DNA
gcgaattccacggcgatcttgccgcccttct

SEQ ID NO: 14 - DNA, 24 bp, synthetic construct
  misc_feature 1..24: note = primer
  source 1..24: mol_type = other DNA
atttctccgtgataggtatcgatg

SEQ ID NO: 15 - DNA, 22 bp, synthetic construct
  misc_feature 1..22: note = primer
  source 1..22: mol_type = other DNA
aacggtttacgttgaaatgtcc